European Patent Application EP 4 692 116 A1, published February 11, 2026. Title: SINGLE-DOMAIN ANTIBODY OF GDF15 AND USE THEREOF. Applicant: KEXING BIOPHARM CO., LTD. Application US. The sequence listing filed with the application follows.

SEQUENCE LISTING (30 sequences)

SEQ ID NO: 1 - protein, 123 aa, synthetic construct
QVQLVESGGGLVQPGGSLRLSCAASGFTLDYYAIGWFRQAPGKGREGVSCISSNDGSTYYSDSVKGRFTTSRDNAKNTVYLQMNSLKPEDTAVYYCAADLTPCPVNPSVDHYWGQGTQVTVSS

SEQ ID NO: 2 - protein, 121 aa, synthetic construct
QLQLVESGGGLVQPGGSLRLSCVASGFTLDDYAIGWFRQAPGKGLEGVSCISSSDESTYYADSVKGRFTISRDNAKNTAYLQMNSLKPEDTAIYYCAADTECPVQVTSMAWGQGTQVTVSS

SEQ ID NO: 3 - protein, 112 aa, synthetic construct
QVQLVESGGGLVQPGGSLRLSCAASGFTIRTYTMSWYRQAPGKERALVAYITPGGPTYHIDSVKGRFTISRNNAENTVYLQMNSLKPEDTAVYYCGNGFGSWGQGTQVTVSS

SEQ ID NO: 4 - protein, 122 aa, synthetic construct
QLQLVESGGGLVQPGGSLRLSCAASGFTLDYYAIGWFRQAPGKGPEAVSCISSSDGSTYYSDSVKGRFTISRDNAKNTVYLQMNSLKPEDTAVYYCAAGEYGSDCPVQVGSWGQGTQVTVSS

SEQ ID NO: 5 - protein, 122 aa, synthetic construct
QVQLVESGGGLVQPGGSLRLACAASGFTLDAYAVGWFRQAPGKNPEGVSCISSSDGSAYYADSVKGRFTISRDNAKNTVYLQMNSLKPGDTAVYYCAADLSCPVQIATFHSRGQGTQVTVSS

SEQ ID NO: 6 - protein, 126 aa, synthetic construct
QLQLVESGGGEVQPGGSLRLSCAASGATLDDLSIGWFRQAPGKGLEGVSCISSSDGSTYYADSVKGRFTISRDNAKNTAYLQMNSLRPEDTAVYYCAADREDCPVQPWGIVAGTSRGQGTQVTVSS

SEQ ID NO: 7 - protein, 5 aa, synthetic construct
YYAIG

SEQ ID NO: 8 - protein, 17 aa, synthetic construct
CISSNDGSTYYSDSVKG

SEQ ID NO: 9 - protein, 14 aa, synthetic construct
DLTPCPVNPSVDHY

SEQ ID NO: 10 - protein, 5 aa, synthetic construct
DYAIG

SEQ ID NO: 11 - protein, 17 aa, synthetic construct
CISSSDESTYYADSVKG

SEQ ID NO: 12 - protein, 12 aa, synthetic construct
DTECPVQVTSMA

SEQ ID NO: 13 - protein, 5 aa, synthetic construct
TYTMS

SEQ ID NO: 14 - protein, 16 aa, synthetic construct
YITPGGPTYHIDSVKG

SEQ ID NO: 15 - protein, 4 aa, synthetic construct
GFGS

SEQ ID NO: 16 - protein, 5 aa, synthetic construct
YYAIG

SEQ ID NO: 17 - protein, 17 aa, synthetic construct
CISSSDGSTYYSDSVKG

SEQ ID NO: 18 - protein, 13 aa, synthetic construct
GEYGSDCPVQVGS

SEQ ID NO: 19 - protein, 5 aa, synthetic construct
AYAVG

SEQ ID NO: 20 - protein, 17 aa, synthetic construct
CISSSDGSAYYADSVKG

SEQ ID NO: 21 - protein, 13 aa, synthetic construct
DLSCPVQIATFHS

SEQ ID NO: 22 - protein, 5 aa, synthetic construct
DLSIG

SEQ ID NO: 23 - protein, 17 aa, synthetic construct
CISSSDGSTYYADSVKG

SEQ ID NO: 24 - protein, 17 aa, synthetic construct
DREDCPVQPWGIVAGTS

SEQ ID NO: 25 - protein, 232 aa, synthetic construct
EPKSADKTHTCPPCPAPELLGGPSVFLFPPKPKDTLMISRTPEVTCVVVDVSHEDPEVKFNWYVDGVEVHNAKTKPREEQYNSTYRVVSVLTVLHQDWLNGKEYKCKVSNKALPAPIEKTISKAKGQPREPQVYTLPPSREEMTKNQVSLTCLVKGFYPSDIAVEWESNGQPENNYKTTPPVLDSDGSFFLYSKLTVDKSRWQQGNVFSCSVMHEALHNHYTQKSLSLSPGK

SEQ ID NO: 26 - protein, 355 aa, synthetic construct
QVQLVESGGGLVQPGGSLRLSCAASGFTLDYYAIGWFRQAPGKGREGVSCISSNDGSTYYSDSVKGRFTTSRDNAKNTVYLQMNSLKPEDTAVYYCAADLTPCPVNPSVDHYWGQGTQVTVSSEPKSADKTHTCPPCPAPELLGGPSVFLFPPKPKDTLMISRTPEVTCVVVDVSHEDPEVKFNWYVDGVEVHNAKTKPREEQYNSTYRVVSVLTVLHQDWLNGKEYKCKVSNKALPAPIEKTISKAKGQPREPQVYTLPPSREEMTKNQVSLTCLVKGFYPSDIAVEWESNGQPENNYKTTPPVLDSDGSFFLYSKLTVDKSRWQQGNVFSCSVMHEALHNHYTQKSLSLSPGK

SEQ ID NO: 27 - protein, 353 aa, synthetic construct
QLQLVESGGGLVQPGGSLRLSCVASGFTLDDYAIGWFRQAPGKGLEGVSCISSSDESTYYADSVKGRFTISRDNAKNTAYLQMNSLKPEDTAIYYCAADTECPVQVTSMAWGQGTQVTVSSEPKSADKTHTCPPCPAPELLGGPSVFLFPPKPKDTLMISRTPEVTCVVVDVSHEDPEVKFNWYVDGVEVHNAKTKPREEQYNSTYRVVSVLTVLHQDWLNGKEYKCKVSNKALPAPIEKTISKAKGQPREPQVYTLPPSREEMTKNQVSLTCLVKGFYPSDIAVEWESNGQPENNYKTTPPVLDSDGSFFLYSKLTVDKSRWQQGNVFSCSVMHEALHNHYTQKSLSLSPGK

SEQ ID NO: 28 - protein, 354 aa, synthetic construct
QLQLVESGGGLVQPGGSLRLSCAASGFTLDYYAIGWFRQAPGKGPEAVSCISSSDGSTYYSDSVKGRFTISRDNAKNTVYLQMNSLKPEDTAVYYCAAGEYGSDCPVQVGSWGQGTQVTVSSEPKSADKTHTCPPCPAPELLGGPSVFLFPPKPKDTLMISRTPEVTCVVVDVSHEDPEVKFNWYVDGVEVHNAKTKPREEQYNSTYRVVSVLTVLHQDWLNGKEYKCKVSNKALPAPIEKTISKAKGQPREPQVYTLPPSREEMTKNQVSLTCLVKGFYPSDIAVEWESNGQPENNYKTTPPVLDSDGSFFLYSKLTVDKSRWQQGNVFSCSVMHEALHNHYTQKSLSLSPGK

SEQ ID NO: 29 - protein, 354 aa, synthetic construct
QVQLVESGGGLVQPGGSLRLACAASGFTLDAYAVGWFRQAPGKNPEGVSCISSSDGSAYYADSVKGRFTISRDNAKNTVYLQMNSLKPGDTAVYYCAADLSCPVQIATFHSRGQGTQVTVSSEPKSADKTHTCPPCPAPELLGGPSVFLFPPKPKDTLMISRTPEVTCVVVDVSHEDPEVKFNWYVDGVEVHNAKTKPREEQYNSTYRVVSVLTVLHQDWLNGKEYKCKVSNKALPAPIEKTISKAKGQPREPQVYTLPPSREEMTKNQVSLTCLVKGFYPSDIAVEWESNGQPENNYKTTPPVLDSDGSFFLYSKLTVDKSRWQQGNVFSCSVMHEALHNHYTQKSLSLSPGK

SEQ ID NO: 30 - protein, 358 aa, synthetic construct
QLQLVESGGGEVQPGGSLRLSCAASGATLDDLSIGWFRQAPGKGLEGVSCISSSDGSTYYADSVKGRFTISRDNAKNTAYLQMNSLRPEDTAVYYCAADREDCPVQPWGIVAGTSRGQGTQVTVSSEPKSADKTHTCPPCPAPELLGGPSVFLFPPKPKDTLMISRTPEVTCVVVDVSHEDPEVKFNWYVDGVEVHNAKTKPREEQYNSTYRVVSVLTVLHQDWLNGKEYKCKVSNKALPAPIEKTISKAKGQPREPQVYTLPPSREEMTKNQVSLTCLVKGFYPSDIAVEWESNGQPENNYKTTPPVLDSDGSFFLYSKLTVDKSRWQQGNVFSCSVMHEALHNHYTQKSLSLSPGK